European Patent Application EP 4 640 823 A1, published October 29, 2025. Title: 柯林斯菌新菌种及其药物组合物. Applicant: 慕恩（广州）生物科技有限公司. The sequence listing filed with the application follows.

SEQUENCE LISTING (3 sequences)

SEQ ID NO: 1 - RNA, 1346 nt, Collinsella sp.
  source 1..1346: mol_type = other RNA
cagtcgtaccaacgagtccatcgtaaggagggaagcgagtggcgaacggctgagtaacacgtgaccaacctgcccggctctcggggatagccgcgggaaaccgcgggtaatacccggcgaacccgcccggacgcatgtccgggcgggcgaagctttcgcggagccggatggggtcgcggcccatcaggtagacggcggggtgacggcccaccgtgcctacaacgggtagccgggttgagagaccgaccggccagattgggactgagacacggcccagactcctacgggaggcagcagtggggaatcttgcgcaatgggggcaaccctgacgcagcgacgccgcgtgcgggacgaaggccttcgggtcgtaaaccgctttcagcagggacgagtcaagacggtacctgcagaagaagccccggctaactacgtgccagcagccgcggtaatacgtagggggcgagcgttatccggattcattgggcgtaaagcgcgcgtaggcggccgcgtaggcggggggtcaaatcccggggctcaaccccggtccgccccccgaaccccgcggctcgggtccggtaggggagggtggaattcccggtgtagcggtggaatgcgcagatatcgggaggaacaccggtggcgaaggcggccctctgggccgagaccgacgctgaggcgcgaaagctgggggagcgaacaggattagataccctggtagtcccagccgtaaacgatggacgctaggtgtgggggggcgatccccccgtgccgcagccaacgcattaagcgtcccgcctggggagtacggccgcaaggctaaaactcaaaggaattgacgggggcccgcacaagcagcggagcatgtggcttaattcgaagcaacgcgaagaaccttaccagggcttgacatgctagtgaagccggggagacccggtggccgagaggagctagcacaggtggtgcatggctgtcgtcagctcgtgtcgtgagatgttgggttaagtcccgcaacgagcgcaacccccgccgcatgttgccagcaggtgaggctgggcacccatgcgggaccgccggcgccaagccggaggagggcggggacgacgtcaagtcatcatgccccttatgccctgggctgcacacgtgctacaatggccggtacagcgggatgcgatggcgcgagccggagcggatccctcaaagccggccccagttcggattgggggctgcaacccgcccccatgaagtcggagttgctagtaatcgcggatcagcatgccgcggtgaatgcgttcccgggccttgtacacaccgcccgtcacaccacccgagtcgtctgcacccgaagc

SEQ ID NO: 2 - DNA, 20 bp, synthetic construct
  source 1..20: mol_type = other DNA
agagtttgatcatggctcag

SEQ ID NO: 3 - DNA, 22 bp, synthetic construct
  source 1..22: mol_type = other DNA
tagggttaccttgttacgactt